European Patent Specification EP 4 006 168 B1, published December 17, 2025. Title: METHOD. Applicant: OXFORD NANOPORE TECHNOLOGIES LIMITED. The sequence listing filed with the application follows.

SEQUENCE LISTING (13 sequences)

SEQ ID NO: 1 - DNA, 558 bp, Artificial sequence
  MS-B1 mutant MspA monomer
atgggtctggataatgaactgagcctggtggacggtcaagatcgtaccctgacggtgcaacaatgggatacctttctgaatggcgtttttccgctggatcgtaatcgcctgacccgtgaatggtttcattccggtcgcgcaaaatatatcgtcgcaggcccgggtgctgacgaattcgaaggcacgctggaactgggttatcagattggctttccgtggtcactgggcgttggtatcaacttctcgtacaccacgccgaatattctgatcaacaatggtaacattaccgcaccgccgtttggcctgaacagcgtgattacgccgaacctgtttccgggtgttagcatctctgcccgtctgggcaatggtccgggcattcaagaagtggcaacctttagtgtgcgcgtttccggcgctaaaggcggtgtcgcggtgtctaacgcccacggtaccgttacgggcgcggccggcggtgtcctgctgcgtccgttcgcgcgcctgattgcctctaccggcgacagcgttacgacctatggcgaaccgtggaatatgaactaa

SEQ ID NO: 2 - protein, 184 aa, Artificial sequence
  MS-B1 mutant MspA monomer
GLDNELSLVDGQDRTLTVQQWDTFLNGVFPLDRNRLTREWFHSGRAKYIVAGPGADEFEGTLELGYQIGFPWSLGVGINFSYTTPNILINNGNITAPPFGLNSVITPNLFPGVSISARLGNGPGIQEVATFSVRVSGAKGGVAVSNAHGTVTGAAGGVLLRPFARLIASTGDSVTTYGEPWNMN

SEQ ID NO: 3 - DNA, 885 bp, Artificial sequence
  alpha-hemolysin-E111N/K147N
atggcagattctgatattaatattaaaaccggtactacagatattggaagcaatactacagtaaaaacaggtgatttagtcacttatgataaagaaaatggcatgcacaaaaaagtattttatagttttatcgatgataaaaatcacaataaaaaactgctagttattagaacaaaaggtaccattgctggtcaatatagagtttatagcgaagaaggtgctaacaaaagtggtttagcctggccttcagcctttaaggtacagttgcaactacctgataatgaagtagctcaaatatctgattactatccaagaaattcgattgatacaaaaaactatatgagtactttaacttatggattcaacggtaatgttactggtgatgatacaggaaaaattggcggccttattggtgcaaatgtttcgattggtcatacactgaactatgttcaacctgatttcaaaacaattttagagagcccaactgataaaaaagtaggctggaaagtgatatttaacaatatggtgaatcaaaattggggaccatacgatcgagattcttggaacccggtatatggcaatcaacttttcatgaaaactagaaatggttctatgaaagcagcagataacttccttgatcctaacaaagcaagttctctattatcttcagggttttcaccagacttcgctacagttattactatggatagaaaagcatccaaacaacaaacaaatatagatgtaatatacgaacgagttcgtgatgattaccaattgcattggacttcaacaaattggaaaggtaccaatactaaagataaatggacagatcgttcttcagaaagatataaaatcgattgggaaaaagaagaaatgacaaattaa

SEQ ID NO: 4 - protein, 293 aa, Artificial sequence
  alpha-hemolysin-E111N/K147N
ADSDINIKTGTTDIGSNTTVKTGDLVTYDKENGMHKKVFYSFIDDKNHNKKLLVIRTKGTIAGQYRVYSEEGANKSGLAWPSAFKVQLQLPDNEVAQISDYYPRNSIDTKNYMSTLTYGFNGNVTGDDTGKIGGLIGANVSIGHTLNYVQPDFKTILESPTDKKVGWKVIFNNMVNQNWGPYDRDSWNPVYGNQLFMKTRNGSMKAADNFLDPNKASSLLSSGFSPDFATVITMDRKASKQQTNIDVIYERVRDDYQLHWTSTNWKGTNTKDKWTDRSSERYKIDWEKEEMTN

SEQ ID NO: 5 - protein, 184 aa, Mycobacterium smegmatis
GLDNELSLVDGQDRTLTVQQWDTFLNGVFPLDRNRLTREWFHSGRAKYIVAGPGADEFEGTLELGYQIGFPWSLGVGINFSYTTPNILIDDGDITAPPFGLNSVITPNLFPGVSISADLGNGPGIQEVATFSVDVSGPAGGVAVSNAHGTVTGAAGGVLLRPFARLIASTGDSVTTYGEPWNMN

SEQ ID NO: 6 - protein, 184 aa, Mycobacterium smegmatis
GLDNELSLVDGQDRTLTVQQWDTFLNGVFPLDRNRLTREWFHSGRAKYIVAGPGADEFEGTLELGYQIGFPWSLGVGINFSYTTPNILIDDGDITGPPFGLESVITPNLFPGVSISADLGNGPGIQEVATFSVDVSGPAGGVAVSNAHGTVTGAAGGVLLRPFARLIASTGDSVTTYGEPWNMN

SEQ ID NO: 7 - protein, 183 aa, Mycobacterium smegmatis
VDNQLSVVDGQGRTLTVQQAETFLNGVFPLDRNRLTREWFHSGRATYHVAGPGADEFEGTLELGYQVGFPWSLGVGINFSYTTPNILIDGGDITQPPFGLDTIITPNLFPGVSISADLGNGPGIQEVATFSVDVKGAKGAVAVSNAHGTVTGAAGGVLLRPFARLIASTGDSVTTYGEPWNMN

SEQ ID NO: 8 - RNA, 90 nt, Artificial sequence
  mRNA sequence analysed in the Examples
guaucuccaucgcugauuagagaaauacaaagaacaaacaaucgggcaccagaacaaaggucguagugcuaaaaaaaaaaaaaaaaaaaa

SEQ ID NO: 9 - DNA, 47 bp, Artificial sequence
  Primer sequence used in the Examples
cccccccccacccccccccacccccccccacccccccccaccccccc

SEQ ID NO: 10 - DNA, 52 bp, Artificial sequence
  Primer sequence used in the Examples
  misc_feature (51)..(51): n is a, c, or g
  misc_feature (52)..(52): n is a, c, g, or t
ggttgtttctgttggtgctgatattgctttttttttttttttttttttttnn

SEQ ID NO: 11 - DNA, 70 bp, Artificial sequence
  cDNA transcribed in the Examples
agcactacgacctttgttctggtgcccgattgtttgttctttgtatttctctaatcagcgatggagatac

SEQ ID NO: 12 - DNA, 28 bp, Artificial sequence
  Tether sequence used in the Examples
gcaatatcagcaccaacagaaacaacct

SEQ ID NO: 13 - protein, 439 aa, Bacteriophage T4
MTFDDLTEGQKNAFNIVMKAIKEKKHHVTINGPAGTGKTTLTKFIIEALISTGETGIILAAPTHAAKKILSKLSGKEASTIHSILKINPVTYEENVLFEQKEVPDLAKCRVLICDEVSMYDRKLFKILLSTIPPWCTIIGIGDNKQIRPVDPGENTAYISPFFTHKDFYQCELTEVKRSNAPIIDVATDVRNGKWIYDKVVDGHGVRGFTGDTALRDFMVNYFSIVKSLDDLFENRVMAFTNKSVDKLNSIIRKKIFETDKDFIVGEIIVMQEPLFKTYKIDGKPVSEIIFNNGQLVRIIEAEYTSTFVKARGVPGEYLIRHWDLTVETYGDDEYYREKIKIISSDEELYKFNLFLGKTAETYKNWNKGGKAPWSDFWDAKSQFSKVKALPASTFHKAQGMSVDRAFIYTPCIHYADVELAQQLLYVGVTRGRYDVFYV